European Patent Specification EP 3 775 272 B1, published July 30, 2025. Title: METHODS, SYSTEMS, AND COMPOSITIONS FOR COUNTING NUCLEIC ACID MOLECULES. Applicant: PROGENITY, INC. The sequence listing filed with the application follows.

SEQUENCE LISTING (7 sequences)

SEQ ID NO: 1 - DNA, 56 bp, Artificial sequence
  Synthetic
agtctaggattcggcgtgggttaaggtggcttccttggccgaagtgcggggaccgc

SEQ ID NO: 2 - DNA, 100 bp, Artifical sequence
  misc_feature (1)..(1): The sequence is circular where position 1 connects to position 100
ccttcgacttcaagagaccatgagttgtgcggtccccgcacttcggccaaggaagccaccatcatcagtagtgtgatggcagcctagcacgggcattagc

SEQ ID NO: 3 - skipped

SEQ ID NO: 4 - DNA, 48 bp, Artifical sequence
gtttcatcagatcctaagccgcacaattgggtgcggcttaggatctga

SEQ ID NO: 5 - DNA, 103 bp, Artificial sequence
  Synthetic
agtctaggattcggcgtgggttaacacgccgaatcctagactactttgatctaggattcggcgtgggttaaggtggcttccttggccgaagtgcggggaccgc

SEQ ID NO: 6 - DNA, 96 bp, Artificial sequence
  Synthetic
ttaacccacgccgaatcctagactcaaagtagtctaggattcggcgtgttaacccacgccgaatcctagactcaaagtagtctaggattcggcgtg

SEQ ID NO: 7 - DNA, 104 bp, Artificial sequence
  Synthetic
agtctaggattcggcgtgggttaacacgccgaatcctagactactttgagtctaggattcggcgtgggttaaggtggcttccttggccgaagtgcggggacccc